European Patent Specification EP 4 031 522 B1, published April 22, 2026. Title: Lipidoids for nucleic acid transfection and use thereof. Applicant: Ustav organicke chemie a biochemie AV CR, v. v. i. The sequence listing filed with the application follows.

SEQUENCE LISTING (10 sequences)

SEQ ID NO: 1 - DNA, 23 bp, artificial
  primer
atcaacatatggtgagcgagctg

SEQ ID NO: 2 - DNA, 26 bp, artificial
  primer
aagaattcctatcatctgtgccccag

SEQ ID NO: 3 - DNA, 21 bp, artificial
  primer
cgagaggagggtctcaaagag

SEQ ID NO: 4 - DNA, 20 bp, artificial
  primer
atttcgggaaggctgctgtc

SEQ ID NO: 5 - DNA, 20 bp, artificial
  primer
aatcccatcaccatcttcca

SEQ ID NO: 6 - DNA, 20 bp, artificial
  primer
tggactccacgacgtactca

SEQ ID NO: 7 - DNA, 20 bp, artificial
  primer
taatacgactcactataggg

SEQ ID NO: 8 - DNA, 19 bp, artificial
  primer
gctagttattgctcagcgg

SEQ ID NO: 9 - DNA, 26 bp, artificial
  primer
taatacgactcactatagaatttact

SEQ ID NO: 10 - DNA, 20 bp, artificial
  primer
ctaatcgccatcttccagca